European Patent Specification EP 3 987 062 B1, published May 21, 2025. Title: DETECTION OF HYPERMETHYLATED GENES FOR DIAGNOSING GASTRIC CANCER. Applicant: UNIVERSITE DE PARIS INSTITUT NATIONAL DE LA SANTE ET DE LA RECHERCHE MEDICALE (INSERM) ASSISTANCE PUBLIQUE-HOPITAUX DE PARIS (AP-HP) Centre National de la Recherche Scientifique (CNRS). The sequence listing filed with the application follows.

SEQUENCE LISTING (21 sequences)

SEQ ID NO: 1 - DNA, 405 bp, homo sapiens
  chr8: 72755783 -72756187
tcgaattcttcccaacgggctgaccctgcccggcgcccaggagcgccctgggtatctcctggctgctctcccgaatccttgcgcgccgcgcccctaccaggttcactgggtgcacgtagccgttctcatagcggtcctcctgcaacagctgccgcaggtgagcgatgtaactggaagccagccggagcgtgtccagcttggagagcttagtgtcggggggcacccagggcaggctggtcttgagcctggagaaggctttgctcagcacgcgcatccgggcacgctcacgggcgttggccgcgttccgctgcgactgcttgcactctgcggctgagcccttggccgggaggggcttcttgccaccaccgcccgcgctaccacctgcgccgccgcccccagccacac

SEQ ID NO: 2 - DNA, 281 bp, homo sapiens
  chr19: 37288170 -37288450
cgcccgcctcggcctcccaaagtgctgggattacaggcgtgagccgccgcgctcggccggccccaaacacttcttattggctaatctggagcaaacctgcatatccattggctgaaagctccgtctattttagggtgactgagagcgtctcttccttctgtgttgcctggaaacggactgttcgcctagtaacatctgatcacgtttcccattggtcaccgtttccggaagcccgctctcccgtttccggaatccccgcaggcgctgggtctgcagatggc

SEQ ID NO: 3 - DNA, 410 bp, homo sapiens
  chr1: 111217406 -111218015
cgcagaaggctgaggcgctcgtccatgcggcggggaagaggcggcagcggtgaggccaggtcgctcctcctcgcgctccccgccctttcgccgcctccgcccccgagccgagcccaccgcctgttgcagccaaagccgcgatgctctgtctgggtctggcgcggtcagccgggctcccgcacggggacgcctcctccctccttctcgcgctctccgccccctcccctgcggggcgcgcgcccgcctccgcgtccccttaggattcccgcccaccgcgcgggcgcgcgtcccgctctcgggggcagccgccgggcctgcatttcttgcagccctcaaggcccctcggtgtcagcgaaagagccctcatgttgtacctcggcgccccgcgggaatgcccacccagcagagcc

SEQ ID NO: 4 - DNA, 702 bp, homo sapiens
  chr8:72755486-72756187
cggccttccctcctttaagaaagggcttgccgattcaaacctgcccgactcagctggattaagttgggcaagggagatttgccgtcagtctgcaacctggtggcagatggagatggaaccaagatttaccctggaagtaggatattagtcaatggctgtcactggggtacaatgttcagaacgatgcaaacagacacggagggttgattcttcttcagggaaatggctggccactcccttgatttgggagaaactaaactggccttctcgttcccagtcccagaacctccacccctttcgaattcttcccaacgggctgaccctgcccggcgcccaggagcgccctgggtatctcctggctgctctcccgaatccttgcgcgccgcgcccctaccaggttcactgggtgcacgtagccgttctcatagcggtcctcctgcaacagctgccgcaggtgagcgatgtaactggaagccagccggagcgtgtccagcttggagagcttagtgtcggggggcacccagggcaggctggtcttgagcctggagaaggctttgctcagcacgcgcatccgggcacgctcacgggcgttggccgcgttccgctgcgactgcttgcactctgcggctgagcccttggccgggaggggcttcttgccaccaccgcccgcgctaccacctgcgccgccgcccccagccacac

SEQ ID NO: 5 - DNA, 641 bp, homo sapiens
  chr19:37288171-37288811
gcccgcctcggcctcccaaagtgctgggattacaggcgtgagccgccgcgctcggccggccccaaacacttcttattggctaatctggagcaaacctgcatatccattggctgaaagctccgtctattttagggtgactgagagcgtctcttccttctgtgttgcctggaaacggactgttcgcctagtaacatctgatcacgtttcccattggtcaccgtttccggaagcccgctctcccgtttccggaatccccgcaggcgctgggtctgcagatggcgtccaggtacacagtggcgagtgtgattccgcagtcttgggctgtttggccaagcgcccgccggacatggtacgccgaagggtcatcggcgtggagtcctcgctttcagcgtccgcggctgggaaatcggccatcgctacggcgggaactgggactcgggctgcgtcccggcccttccacatcggtccaccgcactcgtgggcgcccgcattggtgctgacataatttcctgacctctgacccgtattgtctcgcgattaaaggtaaaaaacggggctttttcatcccactggggtaaaacgcccttttatttctagccaggtgttctgttgcagaacgcctcgaagggagggagtgaccg

SEQ ID NO: 6 - DNA, 610 bp, homo sapiens
  chr1:111217406-111218015
cgcagaaggctgaggcgctcgtccatgcggcggggaagaggcggcagcggtgaggccaggtcgctcctcctcgcgctccccgccctttcgccgcctccgcccccgagccgagcccaccgcctgttgcagccaaagccgcgatgctctgtctgggtctggcgcggtcagccgggctcccgcacggggacgcctcctccctccttctcgcgctctccgccccctcccctgcggggcgcgcgcccgcctccgcgtccccttaggattcccgcccaccgcgcgggcgcgcgtcccgctctcgggggcagccgccgggcctgcatttcttgcagccctcaaggcccctcggtgtcagcgaaagagccctcatgttgtacctcggcgccccgcgggaatgcccacccagcagagccggcccacggggagtcaggctgccggcccgggcccctaggctccgcccgcttctggtcagcgcccctcgcccccggcccgcctggccgcgtcccagtcgccagggttttcggcccgtgggccgggagagctcccgccgcggccccgcgggcgccggccccctggcctccacacccctaggtacagcccggggagggcaggc

SEQ ID NO: 7 - DNA, 21 bp, Artificial Sequence
  forward primer MSC-A1 FP1
cgcgtattcgggtacggttta

SEQ ID NO: 8 - DNA, 20 bp, Artificial Sequence
  reverse primer MSC-AS1 RP1
ctcccgaccaaaaactcaac

SEQ ID NO: 9 - DNA, 20 bp, Artificial Sequence
  forward primer MSC-AS1 er FP
cgtattcgggtacgtttacg

SEQ ID NO: 10 - DNA, 21 bp, Artificial Sequence
  reverse primer MSC-AS1 er RP
ctcccgaccaaaaactcaacc

SEQ ID NO: 11 - DNA, 20 bp, Artificial Sequence
  forward primer ZNF790-AS1 FP
tgttgtttggaaacggattg

SEQ ID NO: 12 - DNA, 23 bp, Artificial Sequence
  reverse primer ZNF790-AS1 RP1
aaaaacgaacttccgaaaacgat

SEQ ID NO: 13 - DNA, 20 bp, Artificial Sequence
  reverse primer ZNF790-AS1 er RP
tgtttggaaacggattgttc

SEQ ID NO: 14 - DNA, 20 bp, Artificial Sequence
  forward primer ZNF790-AS1 er FP
gcctacgaaaattccgaaaa

SEQ ID NO: 15 - DNA, 20 bp, Artificial Sequence
  forward primer KCNA3 FP2
tagcggtgaggttaggtcgt

SEQ ID NO: 16 - DNA, 22 bp, Artificial Sequence
  reverse primer KCNA3 RP3
gcgactttaactacaacaaacg

SEQ ID NO: 17 - DNA, 18 bp, Artificial Sequence
  Probe MSC-AS1: FAM - SEQ ID NO:17 -MGB - NFQ
caaaatacaaacaatcgc

SEQ ID NO: 18 - DNA, 19 bp, Artificial Sequence
  probe MSC-AS1 er : FAM 6 - SEQ ID NO:18 - MGB - NFQ
aaacaatcgcaacgaaacg

SEQ ID NO: 19 - DNA, 23 bp, Artificial Sequence
  probe ZNF790-AS1: FAM - SEQ ID NO:19 - MGB - NFQ
cgtaatcaaatattactaaacga

SEQ ID NO: 20 - DNA, 20 bp, Artificial Sequence
  probe ZNF790-AS1 er: FAM - SEQ ID NO: 20- MGB - NFQ
aaacgaacttccgaaaacga

SEQ ID NO: 21 - DNA, 24 bp, Artificial Sequence
  probe KCNA3: FAM - SEQ ID NO:21 - MGB -NFQ
ctcgagctcgaaaacgaaaacgac